European Patent Specification EP 3 635 009 B1, published February 25, 2026. Title: COMPOSITIONS AND METHODS FOR INTERNALIZING ENZYMES. Applicant: Regeneron Pharmaceuticals, Inc. Baik, Andrew Cygnar, Katherine Schoenherr, Christopher Kyratsous, Christos Wang, Cheng. The sequence listing filed with the application follows.

SEQUENCE LISTING (81 sequences)

SEQ ID NO: 1 - protein, 952 aa, Homo sapiens
MGVRHPPCSHRLLAVCALVSLATAALLGHILLHDFLLVPRELSGSSPVLEETHPAHQQGASRPGPRDAQAHPGRPRAVPTQCDVPPNSRFDCAPDKAITQEQCEARGCCYIPAKQGLQGAQMGQPWCFFPPSYPSYKLENLSSSEMGYTATLTRTTPTFFPKDILTLRLDVMMETENRLHFTIKDPANRRYEVPLETPHVHSRAPSPLYSVEFSEEPFGVIVRRQLDGRVLLNTTVAPLFFADQFLQLSTSLPSQYITGLAEHLSPLMLSTSWTRITLWNRDLAPTPGANLYGSHPFYLALEDGGSAHGVFLLNSNAMDVVLQPSPALSWRSTGGILDVYIFLGPEPKSVVQQYLDVVGYPFMPPYWGLGFHLCRWGYSSTAITRQVVENMTRAHFPLDVQWNDLDYMDSRRDFTFNKDGFRDFPAMVQELHQGGRRYMMIVDPAISSSGPAGSYRPYDEGLRRGVFITNETGQPLIGKVWPGSTAFPDFTNPTALAWWEDMVAEFHDQVPFDGMWIDMNEPSNFIRGSEDGCPNNELENPPYVPGVVGGTLQAATICASSHQFLSTHYNLHNLYGLTEAIASHRALVKARGTRPFVISRSTFAGHGRYAGHWTGDVWSSWEQLASSVPEILQFNLLGVPLVGADVCGFLGNTSEELCVRWTQLGAFYPFMRNHNSLLSLPQEPYSFSEPAQQAMRKALTLRYALLPHLYTLFHQAHVAGETVARPLFLEFPKDSSTWTVDHQLLWGEALLITPVLQAGKAEVTGYFPLGTWYDLQTVPVEALGSLPPPPAAPREPAIHSEGQWVTLPAPLDTINVHLRAGYIIPLQGPGLTTTESRQQPMALAVALTKGGEARGELFWDDGESLEVLERGAYTQVIFLARNNTIVNELVRVTSEGAGLQLQKVTVLGVATAPQQVLSNGVPVSNFTYSPDTKVLDICVSLLMGEQFLVSWC

SEQ ID NO: 2 - protein, 245 aa, Artificial
  synthetic
EVKLVESGGGLVQPGGSLKLSCATSGFTFSDYYMSWVRQTPEKRLEWVAYISSSGGSTYYSDTVKGQFTISRDNAKNTLYLQMSRLKSEDTAMYYCARREDYDGRLTYWGQGTLVTISAGGSGGGGSGGGGSGGDIVLTQSPASLAVSLGQRATISCRASKSVSTSGYSYMNWYQQKPGQPPKVLIYLASKLESGVPARFSGSGSGTDFTLNIHPVEEEDAATYYCQHSRELPYTFGGGTKLEIK

SEQ ID NO: 3 - DNA, 21 bp, Artificial
  synthetic
ggaacccctagtgatggagtt

SEQ ID NO: 4 - DNA, 16 bp, Artificial
  synthetic
cggcctcagtgagcga

SEQ ID NO: 5 - DNA, 21 bp, Artificial
  synthetic
cactccctctctgcgcgctcg

SEQ ID NO: 6 - DNA, 141 bp, Artificial
  synthetic
cctgcaggcagctgcgcgctcgctcgctcactgaggccgcccgggcaaagcccgggcgtcgggcgacctttggtcgcccggcctcagtgagcgagcgagcgcgcagagagggagtggccaactccatcactaggggttcct

SEQ ID NO: 7 - DNA, 141 bp, Artificial
  synthetic
aggaacccctagtgatggagttggccactccctctctgcgcgctcgctcgctcactgaggccgggcgaccaaaggtcgcccgacgcccgggctttgcccgggcggcctcagtgagcgagcgagcgcgcagctgcctgcagg

SEQ ID NO: 8 - DNA, 224 bp, Artificial
  synthetic
gtctgtctgcacatttcgtagagcgagtgttccgatactctaatctccctaggcaaggttcatatttgtgtaggttacttattctccttttgttgactaagtcaataatcagaatcagcaggtttggagtcagcttggcagggatcagcagcctgggttggaaggagggggtataaaagccccttcaccaggagaagccgtcacacagatccacaagctcctga

SEQ ID NO: 9 - DNA, 72 bp, Artificial
  synthetic
gggggaggctgctggtgaatattaaccaaggtcaccccagttatcggaggagcaaacaggggctaagtccac

SEQ ID NO: 10 - protein, 1133 aa, Artificial
  synthetic
EVKLVESGGGLVQPGGSLKLSCATSGFTFSDYYMSWVRQTPEKRLEWVAYISSSGGSTYYSDTVKGQFTISRDNAKNTLYLQMSRLKSEDTAMYYCARREDYDGRLTYWGQGTLVTISAGGSGGGGSGGGGSGGDIVLTQSPASLAVSLGQRATISCRASKSVSTSGYSYMNWYQQKPGQPPKVLIYLASKLESGVPARFSGSGSGTDFTLNIHPVEEEDAATYYCQHSRELPYTFGGGTKLEIKGGGGSAHPGRPRAVPTQCDVPPNSRFDCAPDKAITQEQCEARGCCYIPAKQGLQGAQMGQPWCFFPPSYPSYKLENLSSSEMGYTATLTRTTPTFFPKDILTLRLDVMMETENRLHFTIKDPANRRYEVPLETPHVHSRAPSPLYSVEFSEEPFGVIVRRQLDGRVLLNTTVAPLFFADQFLQLSTSLPSQYITGLAEHLSPLMLSTSWTRITLWNRDLAPTPGANLYGSHPFYLALEDGGSAHGVFLLNSNAMDVVLQPSPALSWRSTGGILDVYIFLGPEPKSVVQQYLDVVGYPFMPPYWGLGFHLCRWGYSSTAITRQVVENMTRAHFPLDVQWNDLDYMDSRRDFTFNKDGFRDFPAMVQELHQGGRRYMMIVDPAISSSGPAGSYRPYDEGLRRGVFITNETGQPLIGKVWPGSTAFPDFTNPTALAWWEDMVAEFHDQVPFDGMWIDMNEPSNFIRGSEDGCPNNELENPPYVPGVVGGTLQAATICASSHQFLSTHYNLHNLYGLTEAIASHRALVKARGTRPFVISRSTFAGHGRYAGHWTGDVWSSWEQLASSVPEILQFNLLGVPLVGADVCGFLGNTSEELCVRWTQLGAFYPFMRNHNSLLSLPQEPYSFSEPAQQAMRKALTLRYALLPHLYTLFHQAHVAGETVARPLFLEFPKDSSTWTVDHQLLWGEALLITPVLQAGKAEVTGYFPLGTWYDLQTVPVEALGSLPPPPAAPREPAIHSEGQWVTLPAPLDTINVHLRAGYIIPLQGPGLTTTESRQQPMALAVALTKGGEARGELFWDDGESLEVLERGAYTQVIFLARNNTIVNELVRVTSEGAGLQLQKVTVLGVATAPQQVLSNGVPVSNFTYSPDTKVLDICVSLLMGEQFLVSWC

SEQ ID NO: 11 - DNA, 3489 bp, Artificial
  synthetic
atgcacagacctagacgtcgtggaactcgtccacctccactggcactgctcgctgctctcctcctggctgcacgtggtgctgatgcagaagtgaagctggtggagtctgggggaggcttagtgcagcctggagggtccctgaaactctcctgtgcaacctctggattcactttcagtgactattacatgtcttgggttcgccagactccagagaagaggctggagtgggtcgcatatattagtagtagtggtggtagcacctattattcagacactgtaaagggccaattcaccatctccagagacaatgccaagaacaccctgtacctgcaaatgagccgtctgaagtctgaggacacagccatgtattactgtgcaagacgagaagattacgacggaagacttacttactggggccaagggactctggtcaccatctctgcaggaggaagtggtggaggcgggtcaggaggtggcgggagcggcggtgacattgtgctgacacagtctcctgcttccttagctgtatctctggggcagagggccaccatctcctgcagggccagcaaaagtgtcagtacatctggttatagttatatgaactggtaccaacagaaaccaggacagccacccaaagtcctcatctatcttgcatccaaactagaatctggggtccctgccaggttcagtggcagtgggtcagggacagacttcaccctcaacatccatcctgtggaggaggaggatgctgcaacctattactgtcagcacagtagggagcttccgtacacgttcggaggggggaccaaactggaaataaaaggtggtggcggttcagcacaccccggccgtcccagagcagtgcccacacagtgcgacgtcccccccaacagccgcttcgattgcgcccctgacaaggccatcacccaggaacagtgcgaggcccgcggctgttgctacatccctgcaaagcaggggctgcagggagcccagatggggcagccctggtgcttcttcccacccagctaccccagctacaagctggagaacctgagctcctctgaaatgggctacacggccaccctgacccgtaccacccccaccttcttccccaaggacatcctgaccctgcggctggacgtgatgatggagactgagaaccgcctccacttcacgatcaaagatccagctaacaggcgctacgaggtgcccttggagaccccgcatgtccacagccgggcaccgtccccactctacagcgtggagttctccgaggagcccttcggggtgatcgtgcgccggcagctggacggccgcgtgctgctgaacacgacggtggcgcccctgttctttgcggaccagttccttcagctgtccacctcgctgccctcgcagtatatcacaggcctcgccgagcacctcagtcccctgatgctcagcaccagctggaccaggatcaccctgtggaaccgggaccttgcgcccacgcccggtgcgaacctctacgggtctcaccctttctacctggcgctggaggacggcgggtcggcacacggggtgttcctgctaaacagcaatgccatggatgtggtcctgcagccgagccctgcccttagctggaggtcgacaggtgggatcctggatgtctacatcttcctgggcccagagcccaagagcgtggtgcagcagtacctggacgttgtgggatacccgttcatgccgccatactggggcctgggcttccacctgtgccgctggggctactcctccaccgctatcacccgccaggtggtggagaacatgaccagggcccacttccccctggacgtccagtggaacgacctggactacatggactcccggagggacttcacgttcaacaaggatggcttccgggacttcccggccatggtgcaggagctgcaccagggcggccggcgctacatgatgatcgtggatcctgccatcagcagctcgggccctgccgggagctacaggccctacgacgagggtctgcggaggggggttttcatcaccaacgagaccggccagccgctgattgggaaggtatggcccgggtccactgccttccccgacttcaccaaccccacagccctggcctggtgggaggacatggtggctgagttccatgaccaggtgcccttcgacggcatgtggattgacatgaacgagccttccaacttcatcaggggctctgaggacggctgccccaacaatgagctggagaacccaccctacgtgcctggggtggttggggggaccctccaggcggccaccatctgtgcctccagccaccagtttctctccacacactacaacctgcacaacctctacggcctgaccgaagccatcgcctcccacagggcgctggtgaaggctcgggggacacgcccatttgtgatctcccgctcgacctttgctggccacggccgatacgccggccactggacgggggacgtgtggagctcctgggagcagctcgcctcctccgtgccagaaatcctgcagtttaacctgctgggggtgcctctggtcggggccgacgtctgcggcttcctgggcaacacctcagaggagctgtgtgtgcgctggacccagctgggggccttctaccccttcatgcggaaccacaacagcctgctcagtctgccccaggagccgtacagcttcagcgagccggcccagcaggccatgaggaaggccctcaccctgcgctacgcactcctcccccacctctacacactgttccaccaggcccacgtcgcgggggagaccgtggcccggcccctcttcctggagttccccaaggactctagcacctggactgtggaccaccagctcctgtggggggaggccctgctcatcaccccagtgctccaggccgggaaggccgaagtgactggctacttccccttgggcacatggtacgacctgcagacggtgccagtagaggcccttggcagcctcccacccccacctgcagctccccgtgagccagccatccacagcgaggggcagtgggtgacgctgccggcccccctggacaccatcaacgtccacctccgggctgggtacatcatccccctgcagggccctggcctcacaaccacagagtcccgccagcagcccatggccctggctgtggccctgaccaagggtggggaggcccgaggggagctgttctgggacgatggagagagcctggaagtgctggagcgaggggcctacacacaggtcatcttcctggccaggaataacacgatcgtgaatgagctggtacgtgtgaccagtgagggagctggcctgcagctgcagaaggtgactgtcctgggcgtggccacggcgccccagcaggtcctctccaacggtgtccctgtctccaacttcacctacagccccgacaccaaggtcctggacatctgtgtctcgctgttgatgggagagcagtttctcgtcagctggtgttag

SEQ ID NO: 12 - DNA, 2859 bp, Homo sapiens
atgggagtgaggcacccgccctgctcccaccggctcctggccgtctgcgccctcgtgtccttggcaaccgctgcactcctggggcacatcctactccatgatttcctgctggttccccgagagctgagtggctcctccccagtcctggaggagactcacccagctcaccagcagggagccagcagaccagggccccgggatgcccaggcacaccccggccgtcccagagcagtgcccacacagtgcgacgtcccccccaacagccgcttcgattgcgcccctgacaaggccatcacccaggaacagtgcgaggcccgcggctgttgctacatccctgcaaagcaggggctgcagggagcccagatggggcagccctggtgcttcttcccacccagctaccccagctacaagctggagaacctgagctcctctgaaatgggctacacggccaccctgacccgtaccacccccaccttcttccccaaggacatcctgaccctgcggctggacgtgatgatggagactgagaaccgcctccacttcacgatcaaagatccagctaacaggcgctacgaggtgcccttggagaccccgcatgtccacagccgggcaccgtccccactctacagcgtggagttctccgaggagcccttcggggtgatcgtgcgccggcagctggacggccgcgtgctgctgaacacgacggtggcgcccctgttctttgcggaccagttccttcagctgtccacctcgctgccctcgcagtatatcacaggcctcgccgagcacctcagtcccctgatgctcagcaccagctggaccaggatcaccctgtggaaccgggaccttgcgcccacgcccggtgcgaacctctacgggtctcaccctttctacctggcgctggaggacggcgggtcggcacacggggtgttcctgctaaacagcaatgccatggatgtggtcctgcagccgagccctgcccttagctggaggtcgacaggtgggatcctggatgtctacatcttcctgggcccagagcccaagagcgtggtgcagcagtacctggacgttgtgggatacccgttcatgccgccatactggggcctgggcttccacctgtgccgctggggctactcctccaccgctatcacccgccaggtggtggagaacatgaccagggcccacttccccctggacgtccagtggaacgacctggactacatggactcccggagggacttcacgttcaacaaggatggcttccgggacttcccggccatggtgcaggagctgcaccagggcggccggcgctacatgatgatcgtggatcctgccatcagcagctcgggccctgccgggagctacaggccctacgacgagggtctgcggaggggggttttcatcaccaacgagaccggccagccgctgattgggaaggtatggcccgggtccactgccttccccgacttcaccaaccccacagccctggcctggtgggaggacatggtggctgagttccatgaccaggtgcccttcgacggcatgtggattgacatgaacgagccttccaacttcatcaggggctctgaggacggctgccccaacaatgagctggagaacccaccctacgtgcctggggtggttggggggaccctccaggcggccaccatctgtgcctccagccaccagtttctctccacacactacaacctgcacaacctctacggcctgaccgaagccatcgcctcccacagggcgctggtgaaggctcgggggacacgcccatttgtgatctcccgctcgacctttgctggccacggccgatacgccggccactggacgggggacgtgtggagctcctgggagcagctcgcctcctccgtgccagaaatcctgcagtttaacctgctgggggtgcctctggtcggggccgacgtctgcggcttcctgggcaacacctcagaggagctgtgtgtgcgctggacccagctgggggccttctaccccttcatgcggaaccacaacagcctgctcagtctgccccaggagccgtacagcttcagcgagccggcccagcaggccatgaggaaggccctcaccctgcgctacgcactcctcccccacctctacacactgttccaccaggcccacgtcgcgggggagaccgtggcccggcccctcttcctggagttccccaaggactctagcacctggactgtggaccaccagctcctgtggggggaggccctgctcatcaccccagtgctccaggccgggaaggccgaagtgactggctacttccccttgggcacatggtacgacctgcagacggtgccagtagaggcccttggcagcctcccacccccacctgcagctccccgtgagccagccatccacagcgaggggcagtgggtgacgctgccggcccccctggacaccatcaacgtccacctccgggctgggtacatcatccccctgcagggccctggcctcacaaccacagagtcccgccagcagcccatggccctggctgtggccctgaccaagggtggggaggcccgaggggagctgttctgggacgatggagagagcctggaagtgctggagcgaggggcctacacacaggtcatcttcctggccaggaataacacgatcgtgaatgagctggtacgtgtgaccagtgagggagctggcctgcagctgcagaaggtgactgtcctgggcgtggccacggcgccccagcaggtcctctccaacggtgtccctgtctccaacttcacctacagccccgacaccaaggtcctggacatctgtgtctcgctgttgatgggagagcagtttctcgtcagctggtgttag

SEQ ID NO: 13 - DNA, 354 bp, Homo sapiens
caggtgcagctgcaggagtcgggccccggactgatgaagccttcggagaccctgtccctcacctgcactgtctctggtggctccttcagcagttactattggaactggatccggcagtccccagggaagggactggagtggattgggtatatccgttatagtggggacaccaactacaagccctccctcaagagtcgattcaccatatcaattgacacgtccaagaaccttttctccctgaggctgaaatctgtgaccgctgcggacacggccgtgtattactgtgcgaggatgggactggggagtgatgcttttgatatctggggccaagggacaatggtcaccgtctcttca

SEQ ID NO: 14 - protein, 118 aa, Homo sapiens
QVQLQESGPGLMKPSETLSLTCTVSGGSFSSYYWNWIRQSPGKGLEWIGYIRYSGDTNYKPSLKSRFTISIDTSKNLFSLRLKSVTAADTAVYYCARMGLGSDAFDIWGQGTMVTVSS

SEQ ID NO: 15 - DNA, 24 bp, Homo sapiens
ggtggctccttcagcagttactat

SEQ ID NO: 16 - protein, 8 aa, Homo sapiens
GGSFSSYY

SEQ ID NO: 17 - DNA, 21 bp, Homo sapiens
atccgttatagtggggacacc

SEQ ID NO: 18 - protein, 7 aa, Homo sapiens
IRYSGDT

SEQ ID NO: 19 - DNA, 36 bp, Homo sapiens
gcgaggatgggactggggagtgatgcttttgatatc

SEQ ID NO: 20 - protein, 12 aa, Homo sapiens
ARMGLGSDAFDI

SEQ ID NO: 21 - DNA, 324 bp, Homo sapiens
gaaattgtgttgacgcagtctccaggcaccctgtctttgtctccaggggaaagagccaccctctcctgcagggccagtcagagtgttaacaacaattatttagcctggtaccagcagaaacctggccaggctcccaggctcctcatctatggtgtattcaacagggccactaacatcccagacaggttcagtggcagtgggtctgggacagatttcactctcaccatcagcagactggagcctgaagattttgcagtgtattactgtcagcagtatggtagttcaccttggacgttcggccaagggaccaaggtggaaatcaaa

SEQ ID NO: 22 - protein, 108 aa, Homo sapiens
EIVLTQSPGTLSLSPGERATLSCRASQSVNNNYLAWYQQKPGQAPRLLIYGVFNRATNIPDRFSGSGSGTDFTLTISRLEPEDFAVYYCQQYGSSPWTFGQGTKVEIK

SEQ ID NO: 23 - DNA, 21 bp, Homo sapiens
cagagtgttaacaacaattat

SEQ ID NO: 24 - protein, 7 aa, Homo sapiens
QSVNNNY

SEQ ID NO: 25 - DNA, 9 bp, Homo sapiens
ggtgtattc

SEQ ID NO: 26 - protein, 3 aa, Homo sapiens
GVF

SEQ ID NO: 27 - DNA, 27 bp, Homo sapiens
cagcagtatggtagttcaccttggacg

SEQ ID NO: 28 - protein, 9 aa, Homo sapiens
QQYGSSPWT

SEQ ID NO: 29 - DNA, 354 bp, Homo sapiens
caggtgcagctgcaggagtcgggcccaagactggtgaagccttcggagaccctgtccctcacctgcattgtctctggtggctccatcagtaatttctactggaactggatccggcagtccccagggaagggactggaatggattggatatttcttttacactgggactatcgactacaacccctccctcaagagtcgagtcaccatatcactggacacgtccaagaaccagttctccctgaacctgcgtcttctgaccgccgcagacgcggccgtttattattgtgcgaggatggggctgggggctaatgcttttgacatctggggccacgggacaatggtcaccgtctcttca

SEQ ID NO: 30 - protein, 118 aa, Homo sapiens
QVQLQESGPRLVKPSETLSLTCIVSGGSISNFYWNWIRQSPGKGLEWIGYFFYTGTIDYNPSLKSRVTISLDTSKNQFSLNLRLLTAADAAVYYCARMGLGANAFDIWGHGTMVTVSS

SEQ ID NO: 31 - DNA, 24 bp, Homo sapiens
ggtggctccatcagtaatttctac

SEQ ID NO: 32 - protein, 8 aa, Homo sapiens
GGSISNFY

SEQ ID NO: 33 - DNA, 21 bp, Homo sapiens
ttcttttacactgggactatc

SEQ ID NO: 34 - protein, 7 aa, Homo sapiens
FFYTGTI

SEQ ID NO: 35 - DNA, 36 bp, Homo sapiens
gcgaggatggggctgggggctaatgcttttgacatc

SEQ ID NO: 36 - protein, 12 aa, Homo sapiens
ARMGLGANAFDI

SEQ ID NO: 37 - DNA, 324 bp, Homo sapiens
gaaattgtgttgacgcagtctccaggcaccctgtctttgtctcctggagaaagagccaccctctcctgcagggccagtcagcatgttagcagcaactacttagcctggtaccagcagaaacctggccaggctcccaggctcctcatctatggtggatccagcagggccactggcatcccagacaggttcagtggcagtgggtctgggacagacttcactctcaccatcagcagactggagcctgcagattttgcagtgttttactgtcagcagtatggtaactcaccttggacgttcggccaagggaccaaggtggaaatgaaa

SEQ ID NO: 38 - protein, 108 aa, Homo sapiens
EIVLTQSPGTLSLSPGERATLSCRASQHVSSNYLAWYQQKPGQAPRLLIYGGSSRATGIPDRFSGSGSGTDFTLTISRLEPADFAVFYCQQYGNSPWTFGQGTKVEMK

SEQ ID NO: 39 - DNA, 21 bp, Homo sapiens
cagcatgttagcagcaactac

SEQ ID NO: 40 - protein, 7 aa, Homo sapiens
QHVSSNY

SEQ ID NO: 41 - DNA, 9 bp, Homo sapiens
ggtggatcc

SEQ ID NO: 42 - protein, 3 aa, Homo sapiens
GGS

SEQ ID NO: 43 - DNA, 27 bp, Homo sapiens
cagcagtatggtaactcaccttggacg

SEQ ID NO: 44 - protein, 9 aa, Homo sapiens
QQYGNSPWT

SEQ ID NO: 45 - DNA, 351 bp, Homo sapiens
caggtgcaactacaggagtcgggcccaaaggtggtgaagccttcggagaccctgtccctcacctgcactgtctctggtggctccatcagtagttactactggaattggatccgccagtccccagggaagggactggagtggattggatataccaaaagagggtataccgactacaacccctccctcaggagtcgcgtcactatatcagaagacacgtccaagaaccagttctccctgaggatcagctctgtgaccgccgcagacacggccgtatattactgtgcacaaatggggtggggatcccatgcttttgacatgtggggccaagggacaatggtcgccgtctcttca

SEQ ID NO: 46 - protein, 117 aa, Homo sapiens
QVQLQESGPKVVKPSETLSLTCTVSGGSISSYYWNWIRQSPGKGLEWIGYTKRGYTDYNPSLRSRVTISEDTSKNQFSLRISSVTAADTAVYYCAQMGWGSHAFDMWGQGTMVAVSS

SEQ ID NO: 47 - DNA, 24 bp, Homo sapiens
ggtggctccatcagtagttactac

SEQ ID NO: 48 - protein, 8 aa, Homo sapiens
GGSISSYY

SEQ ID NO: 49 - DNA, 18 bp, Homo sapiens
accaaaagagggtatacc

SEQ ID NO: 50 - protein, 6 aa, Homo sapiens
TKRGYT

SEQ ID NO: 51 - DNA, 36 bp, Homo sapiens
gcacaaatggggtggggatcccatgcttttgacatg

SEQ ID NO: 52 - protein, 12 aa, Homo sapiens
AQMGWGSHAFDM

SEQ ID NO: 53 - DNA, 324 bp, Homo sapiens
gaaattgtgttgacgcagtctccaggcaccctgtctttgtctccaggggaaagagccaccctctcctgcagggccagtcagagtgttagcagcagctacttagcctggtaccagcagaaacctggccaggctcccaggctcctcatctatggtgcatccagcagggccactggcatcccagacaggttcagtggcagtgggtctgggacagacttcactctcaccatcagcagactggagcctgaagattttgcagtgtattactgtcagcagtatggtagctcaccttggacgttcggccaagggaccaaggtggaaatcaaa

SEQ ID NO: 54 - protein, 108 aa, Homo sapiens
EIVLTQSPGTLSLSPGERATLSCRASQSVSSSYLAWYQQKPGQAPRLLIYGASSRATGIPDRFSGSGSGTDFTLTISRLEPEDFAVYYCQQYGSSPWTFGQGTKVEIK

SEQ ID NO: 55 - DNA, 21 bp, Homo sapiens
cagagtgttagcagcagctac

SEQ ID NO: 56 - protein, 7 aa, Homo sapiens
QSVSSSY

SEQ ID NO: 57 - DNA, 9 bp, Homo sapiens
ggtgcatcc

SEQ ID NO: 58 - protein, 3 aa, Homo sapiens
GAS

SEQ ID NO: 59 - DNA, 27 bp, Homo sapiens
cagcagtatggtagctcaccttggacg

SEQ ID NO: 60 - protein, 9 aa, Homo sapiens
QQYGSSPWT

SEQ ID NO: 61 - DNA, 351 bp, Homo sapiens; identical to SEQ ID NO: 45

SEQ ID NO: 62 - protein, 117 aa, Homo sapiens; identical to SEQ ID NO: 46

SEQ ID NO: 63 - DNA, 24 bp, Homo sapiens
ggtggctccatcagtagttactac

SEQ ID NO: 64 - protein, 8 aa, Homo sapiens
GGSISSYY

SEQ ID NO: 65 - DNA, 18 bp, Homo sapiens
accaaaagagggtatacc

SEQ ID NO: 66 - protein, 6 aa, Homo sapiens
TKRGYT

SEQ ID NO: 67 - DNA, 36 bp, Homo sapiens; identical to SEQ ID NO: 51

SEQ ID NO: 68 - protein, 12 aa, Homo sapiens
AQMGWGSHAFDM

SEQ ID NO: 69 - DNA, 324 bp, Homo sapiens
gaaattgtgttgacgcagtctccaggcaccctgtctttgtctccaggggaaagagccaccctctcctgcagggccagtcagagtgttaatagtaggtacttagcctggtaccagcagaaacctggccaggctcccaggctcctcatctatggtgcatccagcagggccactggcatcccagacaggtgcagtggcagtgggtccgggacagacttcactctcaccatcagcagactggagcctgaagattttgcagtgtattactgtcagcagtatggtagctcaccttggacgttcggccaggggaccaaggtggaaatcaaa

SEQ ID NO: 70 - protein, 108 aa, Homo sapiens
EIVLTQSPGTLSLSPGERATLSCRASQSVNSRYLAWYQQKPGQAPRLLIYGASSRATGIPDRCSGSGSGTDFTLTISRLEPEDFAVYYCQQYGSSPWTFGQGTKVEIK

SEQ ID NO: 71 - DNA, 21 bp, Homo sapiens
cagagtgttaatagtaggtac

SEQ ID NO: 72 - protein, 7 aa, Homo sapiens
QSVNSRY

SEQ ID NO: 73 - DNA, 9 bp, Homo sapiens
ggtgcatcc

SEQ ID NO: 74 - protein, 3 aa, Homo sapiens
GAS

SEQ ID NO: 75 - DNA, 27 bp, Homo sapiens
cagcagtatggtagctcaccttggacg

SEQ ID NO: 76 - protein, 9 aa, Homo sapiens
QQYGSSPWT

SEQ ID NO: 77 - protein, 238 aa, Homo sapiens
MAVEGGMKCVKFLLYVLLLAFCACAVGLIAVGVGAQLVLSQTIIQGATPGSLLPVVIIAVGVFLFLVAFVGCCGACKENYCLMITFAIFLSLIMLVEVAAAIAGYVFRDKVMSEFNNNFRQQMENYPKNNHTASILDRMQADFKCCGAANYTDWEKIPSMSKNRVPDSCCINVTVGCGINFNEKAIHKEGCVEKIGGWLRKNVLVVAAAALGIAFVEVLGIVFACCLVKSIRSGYEVM

SEQ ID NO: 78 - protein, 917 aa, Homo sapiens
LLVPRELSGSSPVLEETHPAHQQGASRPGPRDAQAHPGRPRAVPTQCDVPPNSRFDCAPDKAITQEQCEARGCCYIPAKQGLQGAQMGQPWCFFPPSYPSYKLENLSSSEMGYTATLTRTTPTFFPKDILTLRLDVMMETENRLHFTIKDPANRRYEVPLETPHVHSRAPSPLYSVEFSEEPFGVIVRRQLDGRVLLNTTVAPLFFADQFLQLSTSLPSQYITGLAEHLSPLMLSTSWTRITLWNRDLAPTPGANLYGSHPFYLALEDGGSAHGVFLLNSNAMDVVLQPSPALSWRSTGGILDVYIFLGPEPKSVVQQYLDVVGYPFMPPYWGLGFHLCRWGYSSTAITRQVVENMTRAHFPLDVQWNDLDYMDSRRDFTFNKDGFRDFPAMVQELHQGGRRYMMIVDPAISSSGPAGSYRPYDEGLRRGVFITNETGQPLIGKVWPGSTAFPDFTNPTALAWWEDMVAEFHDQVPFDGMWIDMNEPSNFIRGSEDGCPNNELENPPYVPGVVGGTLQAATICASSHQFLSTHYNLHNLYGLTEAIASHRALVKARGTRPFVISRSTFAGHGRYAGHWTGDVWSSWEQLASSVPEILQFNLLGVPLVGADVCGFLGNTSEELCVRWTQLGAFYPFMRNHNSLLSLPQEPYSFSEPAQQAMRKALTLRYALLPHLYTLFHQAHVAGETVARPLFLEFPKDSSTWTVDHQLLWGEALLITPVLQAGKAEVTGYFPLGTWYDLQTVPVEALGSLPPPPAAPREPAIHSEGQWVTLPAPLDTINVHLRAGYIIPLQGPGLTTTESRQQPMALAVALTKGGEARGELFWDDGESLEVLERGAYTQVIFLARNNTIVNELVRVTSEGAGLQLQKVTVLGVATAPQQVLSNGVPVSNFTYSPDTKVLDICVSLLMGEQFLVSWC

SEQ ID NO: 79 - protein, 1128 aa, Artificial Sequence
  scFv_H4H123450(VH-linker-VL)_linker_GAA
QVQLQESGPKVVKPSETLSLTCTVSGGSISSYYWNWIRQSPGKGLEWIGYTKRGYTDYNPSLRSRVTISEDTSKNQFSLRISSVTAADTAVYYCAQMGWGSHAFDMWGQGTMVAVSSGGSGGGGSGGGGSGGEIVLTQSPGTLSLSPGERATLSCRASQSVSSSYLAWYQQKPGQAPRLLIYGASSRATGIPDRFSGSGSGTDFTLTISRLEPEDFAVYYCQQYGSSPWTFGQGTKVEIKGGGGSAHPGRPRAVPTQCDVPPNSRFDCAPDKAITQEQCEARGCCYIPAKQGLQGAQMGQPWCFFPPSYPSYKLENLSSSEMGYTATLTRTTPTFFPKDILTLRLDVMMETENRLHFTIKDPANRRYEVPLETPHVHSRAPSPLYSVEFSEEPFGVIVRRQLDGRVLLNTTVAPLFFADQFLQLSTSLPSQYITGLAEHLSPLMLSTSWTRITLWNRDLAPTPGANLYGSHPFYLALEDGGSAHGVFLLNSNAMDVVLQPSPALSWRSTGGILDVYIFLGPEPKSVVQQYLDVVGYPFMPPYWGLGFHLCRWGYSSTAITRQVVENMTRAHFPLDVQWNDLDYMDSRRDFTFNKDGFRDFPAMVQELHQGGRRYMMIVDPAISSSGPAGSYRPYDEGLRRGVFITNETGQPLIGKVWPGSTAFPDFTNPTALAWWEDMVAEFHDQVPFDGMWIDMNEPSNFIRGSEDGCPNNELENPPYVPGVVGGTLQAATICASSHQFLSTHYNLHNLYGLTEAIASHRALVKARGTRPFVISRSTFAGHGRYAGHWTGDVWSSWEQLASSVPEILQFNLLGVPLVGADVCGFLGNTSEELCVRWTQLGAFYPFMRNHNSLLSLPQEPYSFSEPAQQAMRKALTLRYALLPHLYTLFHQAHVAGETVARPLFLEFPKDSSTWTVDHQLLWGEALLITPVLQAGKAEVTGYFPLGTWYDLQTVPVEALGSLPPPPAAPREPAIHSEGQWVTLPAPLDTINVHLRAGYIIPLQGPGLTTTESRQQPMALAVALTKGGEARGELFWDDGESLEVLERGAYTQVIFLARNNTIVNELVRVTSEGAGLQLQKVTVLGVATAPQQVLSNGVPVSNFTYSPDTKVLDICVSLLMGEQFLVSWC

SEQ ID NO: 80 - protein, 125 aa, Artificial Sequence
  CD63 EC loop 2 MMH
RDKVMSEFNNNFRQQMENYPKNNHTASILDRMQADFKCCGAANYTDWEKIPSMSKNRVPDSCCINVTVGCGINFNEKAIHKEGCVEKIGGWLRKNVLEQKLISEEDLGGEQKLISEEDLHHHHHH

SEQ ID NO: 81 - protein, 324 aa, Artificial Sequence
  CD63 EC loop 2 hFC
RDKVMSEFNNNFRQQMENYPKNNHTASILDRMQADFKCCGAANYTDWEKIPSMSKNRVPDSCCINVTVGCGINFNEKAIHKEGCVEKIGGWLRKNVLDKTHTCPPCPAPELLGGPSVFLFPPKPKDTLMISRTPEVTCVVVDVSHEDPEVKFNWYVDGVEVHNAKTKPREEQYNSTYRVVSVLTVLHQDWLNGKEYKCKVSNKALPAPIEKTISKAKGQPREPQVYTLPPSRDELTKNQVSLTCLVKGFYPSDIAVEWESNGQPENNYKTTPPVLDSDGSFFLYSKLTVDKSRWQQGNVFSCSVMHEALHNHYTQKSLSLSPGK